European Patent Specification EP 3 554 530 B1, published August 23, 2023. Title: Antibacterial Method. Applicant: Norwegian University of Life Sciences. The sequence listing filed with the application follows.

SEQUENCE LISTING (39 sequences)

SEQ ID NO: 1 - protein, 37 aa, Enterococcus sp.
MKFKFNPTGTIVKKLTQYEIAWFKNKHGYYPWEIPRC

SEQ ID NO: 2 - protein, 44 aa, Enterococcus sp.
MLAKIKAMIKKFPNPYTLAAKLTTYEINWYKQQYGRYPWERPVA

SEQ ID NO: 3 - protein, 37 aa, Enterococcus sp.
MIKKFPNPYTLAAKLTTYEINWYKQQYGRYPWERPVA

SEQ ID NO: 4 - protein, 37 aa, Artificial Sequence
  EntK1J97
MKFKFNPTGTIVKKLTQYEINWYKQQYGRYPWERPVA

SEQ ID NO: 5 - protein, 44 aa, Artificial Sequence
  EJ-K1
MLAKIKAMIKKFPNPYTLAAKLTTYEIAWFKNKHGYYPWEIPRC

SEQ ID NO: 6 - DNA, 22 bp, Artificial Sequence
  Primer Ent_F
cgaagtggtcaagtccaatggt

SEQ ID NO: 7 - DNA, 21 bp, Artificial Sequence
  Primer Ent_M
gtgcggattgcgccacttgac

SEQ ID NO: 8 - DNA, 24 bp, Artificial Sequence
  Primer Ent_R
gatgacttaagacttctgcatcat

SEQ ID NO: 9 - DNA, 22 bp, Artificial Sequence
  Primer EF_F
gctcttagcaagatttgatggc

SEQ ID NO: 10 - DNA, 22 bp, Artificial Sequence
  Primer EF_M
cgtccacactgactacctcatc

SEQ ID NO: 11 - DNA, 23 bp, Artificial Sequence
  Primer EF_R
cttagaccgtttcgacagtttgc

SEQ ID NO: 12 - DNA, 21 bp, Artificial Sequence
  Primer EF_R2
tgcaatctgtcgacgtgacac

SEQ ID NO: 13 - DNA, 21 bp, Artificial Sequence
  Primer T1_F
agctagctcaaaggaagaggc

SEQ ID NO: 14 - DNA, 21 bp, Artificial Sequence
  Primer T2_F
tgcaatctgtcgacgtgacac

SEQ ID NO: 15 - DNA, 22 bp, Artificial Sequence
  Primer T3_F
gctcgaacagctaagaatgcct

SEQ ID NO: 16 - DNA, 21 bp, Artificial Sequence
  Primer th009
acgtttgagcaatttccttcc

SEQ ID NO: 17 - DNA, 44 bp, Artificial Sequence
  Primer th010
cacattatccattaaaaatcaaacagcgtttcctccgtcttttg

SEQ ID NO: 18 - DNA, 43 bp, Artificial Sequence
  Primer th011
gtccaaaagcataaggaaagtcgaggaatattatgaaacaaag

SEQ ID NO: 19 - DNA, 21 bp, Artificial Sequence
  Primer th012
catttccaactagaagggctg

SEQ ID NO: 20 - DNA, 47 bp, Artificial Sequence
  Primer ds171
atttatatttattattggaggttcaatgaaaacaattatcacattca

SEQ ID NO: 21 - DNA, 49 bp, Artificial Sequence
  Primer ds172
attgggaagagttacatattagaaattaaaagaaaaagcgttgaatatc

SEQ ID NO: 22 - DNA, 20 bp, Artificial Sequence
  Primer ds87
agcgtttcctccgtcttttg

SEQ ID NO: 23 - DNA, 43 bp, Artificial Sequence
  Primer ds88
caaaagacggaggaaacgcttcgaggaatattatgaaacaaag

SEQ ID NO: 24 - DNA, 24 bp, Artificial Sequence
  Primer Kan484.F
gtttgatttttaatggataatgtg

SEQ ID NO: 25 - DNA, 20 bp, Artificial Sequence
  Primer RpsL41.R
ctttccttatgcttttggac

SEQ ID NO: 26 - DNA, 22 bp, Artificial Sequence
  Primer khb31
ataacaaatccagtagctttgg

SEQ ID NO: 27 - DNA, 25 bp, Artificial Sequence
  Primer khb33
tttctaatatgtaactcttcccaat

SEQ ID NO: 28 - DNA, 23 bp, Artificial Sequence
  Primer khb34
catcggaacctatactcttttag

SEQ ID NO: 29 - DNA, 25 bp, Artificial Sequence
  Primer khb36
tgaacctccaataataaatataaat

SEQ ID NO: 30 - DNA, 44 bp, Artificial Sequence
  Primer 466p1
ggtattcttgtcctcgtagctgaatttggccacttttattttgc

SEQ ID NO: 31 - DNA, 44 bp, Artificial Sequence
  Primer 467p2
gcaaaataaaagtggccaaattcagctacgaggacaagaatacc

SEQ ID NO: 32 - DNA, 46 bp, Artificial Sequence
  Primer 468p1
attcttgtcctcgtacatgcatttggccacttttattttgcaaaac

SEQ ID NO: 33 - DNA, 46 bp, Artificial Sequence
  Primer 469p2
gttttgcaaaataaaagtggccaaatgcatgtacgaggacaagaat

SEQ ID NO: 34 - DNA, 38 bp, Artificial Sequence
  Primer 470p1
gtacatgaatttggcgctttttattttgcaaaacgagc

SEQ ID NO: 35 - DNA, 38 bp, Artificial Sequence
  Primer 471p2
gctcgttttgcaaaataaaaagcgccaaattcatgtac

SEQ ID NO: 36 - DNA, 32 bp, Artificial Sequence
  Primer 472-p1
gaatttggccactttgcttttgcaaaacgagc

SEQ ID NO: 37 - DNA, 32 bp, Artificial Sequence
  Primer 473-p2
gctcgttttgcaaaagcaaagtggccaaattc

SEQ ID NO: 38 - DNA, 50 bp, Artificial Sequence
  Primer 474p1
attcttgtcctcgtagctgcatttggcgccttttattttgcaaaacgagc

SEQ ID NO: 39 - DNA, 50 bp, Artificial Sequence
  Primer 475p2
gctcgttttgcaaaataaaaggcgccaaatgcagctacgaggacaagaat